European Patent Application EP 4 481 040 A2, published December 25, 2024. Title: ENZYMATIC REMOVAL OF CHLOROPHYLL SUBSTRATES FROM TRIACYLGLYCEROL-BASED OILS. Applicant: Bunge Global Innovation, LLC. The sequence listing filed with the application follows.

SEQUENCE LISTING (14 sequences)

SEQ ID NO: 1 - protein, 318 aa, Hordeum vulgare
  REGION 1..318: note = CHL26 putative chlorophyllase
MASAGDVFDHGRHGTSLARVEQAKNTRCSAASRVDADAQAQQSPPKPLLVAAPCDAGEYPVVVFLHGYLCNNYFYSQLIQHVASHGFIVVCPQLYTVSGPDTTSEINSAAAVIDWLAAGLSSKLAPGIRPNLAAVSISGHSRGGKVAFALGLGHAKTSLPLAALIAVDPVDGTGMGNQTPPPILAYKPNAIRVPAPVMVIGTGLGELPRNALFPPCAPLGVSHAAFYDECAAPACHLVARDYGHTDMMDDVTTGAKGLATRALCKSGGARAPMRRFVAGAMVAFLNKWVEGKPEWLDAVREQTVAAPVVLSAVEFRDE

SEQ ID NO: 2 - DNA, 957 bp, synthetic construct
  misc_feature 1..957: note = Codon optimized nucleic acid sequence encoding a putative chlorophyllase from Hordeum vulgare CHL26
  source 1..957: mol_type = other DNA
atggcatcagcaggggacgtatttgatcatggacggcacggaaccagtttggcgagggtagaacaagcgaagaacacccgctgtagcgcagcgtcccgcgtggatgcggacgcccaggctcagcagtcgccgcccaaacccctcctggttgcagccccatgcgacgcaggcgaatacccggtggtcgtattccttcacggctacttgtgcaacaattacttctactcgcagctgatccagcatgtcgcgagccacggcttcattgtagtgtgcccgcagctgtataccgtgtctggtccggatacaaccagtgaaattaatagcgccgctgccgtcatcgactggctcgcggcaggactgtcgtccaagctggccccaggcatccgtccgaacctggccgccgtgagcatcagcggccactcacgcggtggcaaggtggcctttgccctgggtctggggcatgccaagaccagcttgccgctggctgccctgattgccgtggatccagtcgacggcaccgggatgggcaaccaaactccccctccgatcctggcctataagccgaacgccattcgggtccctgctcccgtgatggtgatcggcacaggactgggcgaactgcctcgcaacgcgctgtttccaccttgcgcccccttgggtgtgtcgcacgccgcgttctacgatgagtgtgccgcacccgcatgccacctggttgcccgcgactatggccacaccgacatgatggatgacgtaacaaccggcgccaaaggcctggcaacccgtgcgctgtgcaagagcggtggggcaagagccccgatgcgccgttttgtcgccggcgctatggtggcgttcctgaataagtgggtggagggcaagccggaatggttggacgccgtgcgcgaacagaccgtggctgcaccggtggtcctgtccgccgtagagtttcgcgatgagtaa

SEQ ID NO: 3 - protein, 309 aa, Gossypium raimondii
  REGION 1..309: note = CHL25 putative chlorophyllase
MSAPTSLATNVFGFGSYTTMLQKVESVTTSSMPVPPPKSLLIATPSEAGEFPLLIFLHGYLLYNSFYSQLLQHVASHGFIVIAPQLYIVAGPDTTDEIKSTAAITNWLSKGVLQGLLPPYVRPNLSKLALAGHSRGGKVAFALALQKTMTKLKFSTLIGIDPVDGMDKGKQTPPPVLTYIPHSFDLDMAVMVIGSGLGEVKRNPLFPPCAPKGVNHEDFFKECRKPACHIVAKDYGHLDMLDDETNGFRGRSSYCLCKNGEAREPMRRFVGGVVVASMKAYLNGDNTDLIAIKGHEAAPVELKTIEFLV

SEQ ID NO: 4 - protein, 306 aa, Phoenix dactylifera
  REGION 1..306: note = CHL27 putative chlorophyllase
MASVIINKPSATAASVFDYGKLHVDTIPAKQSDESSPPKDILVVCPKVAGSYTVVLFIQGYLLSNAYYTQLLQHVASHGFILIAPQCIVVSPYSEEDITSAAAVTNWLSDGLQSVLPTGVEANLDKLALAGHSRGGHAAFALALGHAETTLKFSLLMGIDPVAGPSKCCQIPPKILTYEPSSFELEIPVLVLGTGLGSEQKNILFPACAPDGVNHKEFYSECKPPCYHFVVTDYGHLDMLDDTAPKITKCVCKNGTNCREIMRRTTGGIMTAFLKAYLLDLEEDLKAIADPQIAPTKLDPVSYRLE

SEQ ID NO: 5 - protein, 326 aa, Phoenix dactylifera
  REGION 1..326: note = CHL28 putative chlorophyllase
MGLEDIFKEGPLPIQTLTIPAQQRATATGPCCHGRASPMEPTALPPKPLMVILPSQEGDYPVLLYLHGYLLLNSYYSQLLCHIASHGYIAIAPQMYTAAGPDATPEIRDAVAITEWLPTGFAGRLPTHVRPDLQKVAVAGHSRGGKVAFGAALGRATPPPSLPYAAIVGVDPVDGMAAGRQTPPLILGYGDHDFENSIPALVIGSGLGPVRRNPLFPPCAPAGVNHVDFFRECRAPAYHFVATEYGHQDFLDDETGGVRGRATYCLCKNGTAREPMRRFAAGIIVAFLNAWLRNDSADLEDVLDPSRAPVKMEPPEWNLFQKVPTL

SEQ ID NO: 6 - protein, 328 aa, Cucumis sativus
  REGION 1..328: note = CHL29 putative chlorophyllase
MAAVVVDVKGKSKSAAVSSVVDLDPHPYDGVFEKGKFEVGVITKTTDIFSTSKPLLVFTPKTPGLYPAILFFHGFSCYGSFYTDFLTLIASHGYVIAAPQLYVMPTTSEMDEIKSAVDVIKWLSSGLDPLLPTNVKGDLSKLSLLGHSRGGKTAFSLALGWGSPSLPFSAIIGIDPVAGSKFFRPEPQILDPPSQPFKISLPITVVGTGLGPQKATPVTCACAPDGLNHIAFFKKCKPTCAHFVAVNYGHMDILDDNPPGMTGYFTNIACKNGKGPRDLMRKCCSGLVVASLKAYLDNDVSILNAIYDPSIAPTELNPVEVIYKTPSA

SEQ ID NO: 7 - protein, 317 aa, Tarenaya hassleriana
  REGION 1..317: note = CHL30 putative chlorophyllase
MGEESERLGSSAFEPGSLPTTVIKADPSREDPVSPPKPVMIVAPTVAGTYPVVFFFHGFYLRNYFYSDVLSHVASHGFILVAPQLCKLLPPGGQVEVDDAGKVINWAPKYLKSLLPGSVKPSGEDTSLVGHSRGGKTAFAVALGHASTLDPSTKFSALVGIDPVAGSNVCMRTQPHILTYEPESFELDMPVAVVGTGLGPKWNNVMPPCAPDGVNHKEFFNECRPTRAHFVAADYGHMDMLDDDLEGAVGYLAGCLCKKGKLDKSGMRRFVGGIVVAFLKYSVFGDKSEINSIVKDPSLSPARIDPPPQFHEASSFV

SEQ ID NO: 8 - protein, 306 aa, Solanum tuberosum
  REGION 1..306: note = CHL31 putative chlorophyllase
MVHGKASIERNIKMGASSIFEIGNETINTINVKSSSSLPCSLLVFSPTTKGSYPVLLFFHGFMLQPSWYKSLLQHISSHRYIIVAPQFPLINLQEMKNVRKIAEWLINNLKSVVPEKVQPDLEKVAISGHSKGGNTAFAVAFDSSMPLKFSALLGIEPVAGTSTSCLCPPYVLEYIPRIFNQSIPVAVLGAGLSNQSTCCLLQSVAPNGVNHAEFFNESKPPCYYFMAKDYGHADMLEAEGIMAILIRILMKSGKGSKDSMIRAVGGIVVAFLKAYLEGQIDDLNDIVKSPNLAPITLDPVISIKD

SEQ ID NO: 9 - protein, 343 aa, Populus trichocarpa
  REGION 1..343: note = CHL32 putative chlorophyllase
MAAIEDSPTFSSVVTPAAFEIGSLPTTEIPVDPVENDSTAPPGSLLIFRPEEKGTYPVILFHHGTGCQNSWYTDVFKFISSHGYIVVAPQLYGLMPPSGQDELDLAAEVANWLPSGLRCVLPEDIEGDIHNLALAGHSRGGYIAFALALGLADVSLDVDFSALIGVDPVAGTSKTNQMEPKILNYESCSFNFSIPVAIIGTGLGNKPACPIIRQTCAPDGVSHTEIFNECKPPCSHFVTTDYGHMDVLDDDIGLIGEGARAMCKGSRRGVSRDPMRRTVGGVSVAFLEAFFKGNYTDYNKILKSNYFAPTTLDPVQNKSEGTSSSSLSAMSMPATLDWHIDEL

SEQ ID NO: 10 - protein, 318 aa, Vigna radiata
  REGION 1..318: note = CHL33 putative chlorophyllase
MAAIEDSPTFSSVVTPAAFEIGSLPTTEIPVDPVENDSTAPPKPLLIFTPTVPGAYPVILFCHGFFVPNTFYSHLLTHIVSHGFILVAPQLFCKGLPMLEPSEVKFAGKVADWLAEGLQPLLPENVEANLEKLVVSGHSKGGKTAFCVALGYAKTKLKFSALVGIDPVAGTSKYCETNPHILKGVPGSFNLNMPVAVIGSELGPKKGNCCSPPCAPDGMNHKEFFKECKPPSAHFVVARYGHMDMLDDETAGVIGTLLSKCACKNGSGPRDLMRRTIGGLVVAFLRAQLNDHWKDFDAILNPNIAPTQLDNMVYIPAS

SEQ ID NO: 11 - protein, 236 aa, synthetic construct
  REGION 1..236: note = Green fluorescent protein
MTALTEGAKLFEKEIPYITELEGDVEGMKFIIKGEGTGDATTGTIKAKYICTTGDLPVPWATLVSTLSYGVQCFAKYPSHIKDFFKSAMPEGYTQERTISFEGDGVYKTRAMVTYERGSIYNRVTLTGENFKKDGHILRKNVAFQCPPSILYILPDTVNNGIRVEFNQAYDIEGVTEKLVTKCSQMNRPLAGSAAVHIPRYHHITYHTKLSKDRDERRDHMCLVEVVKAVDLDTYQ

SEQ ID NO: 12 - protein, 301 aa, Chlamydomonas reinhardtii
  REGION 1..301: note = P2 pyropheophytinase
MSDDYIKRGDLPTSKWSGRVTLRVDSAMAVPLDVVITYPSSGAAAYPVLVMYNGFQAKAPWYRGIVDHVSSWGYTVVQYTNGGLFPIVVDRVELTYLEPLLTWLETQSADAKSPLYGRADVSRLGTMGHSRGGKLAALQFAGRTDVSGCVLFDPVDGSPMTPESADYPSATKALAAAGRSAGLVGAAITGSCNPVGQNYPKFWGALAPGSWQMVLSQAGHMQFARTGNPFLDWSLDRLCGRGTMMSSDVITYSAAFTVAWFEGIFRPAQSQMGISNFKTWANTQVAARSITFDIKPMQSPQ

SEQ ID NO: 13 - DNA, 21 bp, synthetic construct
  misc_feature 1..21: note = SpeI site and ribosome binding site
  source 1..21: mol_type = other DNA
actagtaggaggtaactaatg

SEQ ID NO: 14 - DNA, 12 bp, synthetic construct
  misc_feature 1..12: note = stop codon and XhoI site
  source 1..12: mol_type = other DNA
tgatgactcgag